European Patent Specification EP 3 340 998 B1, published January 11, 2023. Title: Methods And Compositions For Cells Expressing A Chimeric Intracellular Signaling Molecule. Applicant: The Trustees of the University of Pennsylvania and Wayne State University June, Carl H. Milone, Michael Zhao, Yangbing Lum, Lawrence Thakur, Archana. The sequence listing filed with the application follows.

SEQUENCE LISTING (1 sequence)

SEQ ID NO: 1 - protein, 248 aa, Artificial Sequence
  Artifically generated
MALPVTALLLPLALLLHAARPGSTTTPAPRPPTPAPTIASQPLSLRPEACRPAAGGAVHTRGLDFACDIYIWAPLAGTCGVLLLSLVITLYCSAKRGRKKLLYIFKQPFMRPVQTTQEEDGCSCRFPEEEEGGCELRVKFSRSADAPAYKQGQNQLYNELNLGRREEYDVLDKRRGRDPEMGGKPRRKNPQEGLYNELQKDKMAEAYSEIGMKGERRRGKGHDGLYQGLSTATKDTYDALHMQALPPR